European Patent Application EP 4 560 007 A2, published May 28, 2025. Title: COMPOSITIONS FOR METABOLIC HEALTH. Applicant: International N&H Denmark ApS. The sequence listing filed with the application follows.

SEQUENCE LISTING (6 sequences)

SEQ ID NO: 1 - DNA, 1529 bp, Eubacterium eligens
  source 1..1529: mol_type = genomic DNA
ttatgagagtttgatcctggctcaggatgaacgctggcggcgtgcttaacacatgcaagtcgaacgaagcatttgcaacagatttcttcgggatgaagttgcttatgactgagtggcggacgggtgagtaacgcgtgggtaacctgccttgtactgggggatagcagctggaaacggctggtaataccgcataagcgcacaatgttgcatgacatggtgtgaaaaactccggtggtataagatggacccgcgtctgattagctagttggtgagataacagcccaccaaggcgacgatcagtagccgacctgagagggtgaccggccacattgggactgagacacggcccagactcctacgggaggcagcagtggggaatattgcacaatggaggaaactctgatgcagcgacgccgcgtgagtgaagaagtaattcgttatgtaaagctctatcagcagggaagatagtgacggtacctgactaagaagctccggctaaatacgtgccagcagccgcggtaatacgtatggagcaagcgttatccggatttactgggtgtaaagggagtgtaggtggccatgcaagtcagaagtgaaaatccggggctcaaccccggaactgcttttgaaactgtaaggctagagtgcaggaggggtgagtggaattcctagtgtagcggtgaaatgcgtagatattaggaggaacaccagtggcgaaggcggctcactggactgtaactgacactgaggctcgaaagcgtggggagcaaacaggattagataccctggtagtccacgccgtaaacgatgaatactaggtgtcggggcccataagggcttcggtgccgcagcaaacgcaataagtattccacctggggagtacgttcgcaagaatgaaactcaaaggaattgacggggacccgcacaagcggtggagcatgtggtttaattcgaagcaacgcgaagaaccttaccaagtcttgacatcccactgaccggacagtaatgtgtcctttccttcgggacagtggtgacaggtggtgcatggttgtcgtcagctcgtgtcgtgagatgttgggttaagtcccgcaacgagcgcaacccctatccttagtagccagcagtaagatgggcactctagggagactgccagggataacctggaggaaggtggggatgacgtcaaatcatcatgccccttatgacttgggctacacacgtgctacaatggcgtaaacaaagtgaagcgaagtcgtgaggccaagcaaatcacaaaaataacgtctcagttcggattgtagtctgcaactcgactacatgaagctggaatcgctagtaatcgcagatcagaatgctgcggtgaatacgttcccgggtcttgtacacaccgcccgtcacaccatgggagtcgaaaatgcccgaagtcggtgacctaacgtaagaaggagccgccgaaggcaggtttgataactggggtgaagtcgtaacaaggtagccgtatcggaaggtgcggctggatcacctccttt

SEQ ID NO: 2 - DNA, 1529 bp, Intestinimonas massiliensis
  source 1..1529: mol_type = genomic DNA
tattgagagtttgatcctggctcaggatgaacgctggcggcgtgcttaacacatgcaagtcgaacggaacgccaaggaaagagttttcggacaatggaattggctgtttagtggcggacgggtgagtaacgcgtgagtaacctgccttggagtggggaataacacagtgaaaactgtgctaataccgcatgacatattggtgtcgcatggcgctgatatcaaagatttatcgctctgagatggactcgcgtctgattagatagttggcggggtaacggcccaccaagtcgacgatcagtagccggactgagaggttggccggccacattgggactgagacacggcccagactcctacgggaggcagcagtggggaatattgggcaatgggcgcaagcctgacccagcaacgccgcgtgaaggaagaaggctttcgggttgtaaacttcttttaacagggacgaagtaagtgacggtacctgttgaataagccacggctaactacgtgccagcagccgcggtaatacgtaggtggcaagcgttatccggatttactgggtgtaaagggcgtgtaggcgggactgcaagtcagatgtgaaaactatgggctcaacccatagcctgcatttgaaactgtagttcttgagtgtcggagaggcaatcggaattccgtgtgtagcggtgaaatgcgtagatatacggaggaacaccagtggcgaaggcggattgctggacgataactgacgctgaggcgcgaaagcgtggggagcaaacaggattagataccctggtagtccacgccgtaaacgatggatactaggtgtggggggtctgaccccctccgtgccgcagctaacgcaataagtatcccacctggggagtacgatcgcaaggttgaaactcaaaggaattgacgggggcccgcacaagcggtggagtatgtggtttaattcgaagcaacgcgaagaaccttaccagggcttgacatcctactaacgaaccagagatggattaggtgcccttcggggaaagtagagacaggtggtgcatggttgtcgtcagctcgtgtcgtgagatgttgggttaagtcccgcaacgagcgcaacccttattgttagttgctacgcaagagcactctagcgagactgccgttgacaaaacggaggaaggtggggacgacgtcaaatcatcatgccccttatgtcctgggccacacacgtactacaatggcggttaacagagggaggcaaagccgcgaggcagagcaaacccctaaaagccgtcccagttcggattgcaggctgaaacccgcctgtatgaagtcggaatcgctagtaatcgcggatcagcatgccgcggtgaatacgttcccgggccttgtacacaccgcccgtcacaccatgagagtcgggaacacccgaagtccgtagcctaactgcaaagggggcgcggccgaaggtgggttcgataattggggtgaagtcgtaacaaggtagccgtatcggaaggtgcggctggatcacctccttt

SEQ ID NO: 3 - DNA, 1323 bp, Prevotella copri
  source 1..1323: mol_type = genomic DNA
gagattaaagatttatcggtgatggatggggatgcgtctgattagcttgttggcggggtaacggcccaccaaggcaacgatcagtaggggttctgagaggaaggtcccccacattggaactgagacacggtccaaactcctacgggaggcagcagtgaggaatattggtcaatggacgagagtctgaaccagccaagtagcgtgcaggatgacggccctatgggttgtaaactgcttttataagggaataaagtgagtctcgtgagactttttgcatgtaccttatgaataaggaccggctaattccgtgccagcagccgcggtaatacggaaggtccgggcgttatccggatttattgggtttaaagggagcgtaggccggagattaagcgtgttgtgaaatgtagacgctcaacgtctgcactgcagcgcgaactggtttccttgagtacgcacaaagtgggcggaattcgtggtgtagcggtgaaatgcttagatatcacgaagaactccgattgcgaaggcagctcactggagcgcaactgacgctgaagctcgaaagtgcgggtatcgaacaggattagataccctggtagtccgcacggtaaacgatggatgcccgctgttggtctgaacaggtcagcggccaagcgaaagcattaagcatcccacctggggagtacgccggcaacggtgaaactcaaaggaattgacgggggcccgcacaagcggaggaacatgtggtttaattcgatgatacgcgaggaaccttacccgggcttgaattgcagaggaaggatttggagacaatgacgcccttcggggtctctgtgaaggtgctgcatggttgtcgtcagctcgtgccgtgaggtgtcggcttaagtgccataacgagcgcaacccctctccttagttgccatcaggtcaggctgggcactctggggacactgccaccgtaaggtgtgaggaaggtggggatgacgtcaaatcagcacggcccttacgtccggggctacacacgtgttacaatggcaggtacagagagacggttgtacgtaagtacgatcaaatccttaaagcctgtctcagttcggactggggtctgcaacccgaccccacgaagctggattcgctagtaatcgcgcatcagccatggcgcggtgaatacgttcccgggccttgtacacaccgcccgtcaagccatgaaagccgggggcgcctaaagtccgtgaccgtaaggagcggcctagggcgaaactggtaattggggctaagtcgtaacaaggtagccgtaccggaaggtgcggctggaacacctccttt

SEQ ID NO: 4 - DNA, 18 bp, synthetic construct
  misc_feature 1..18: note = Primer
  source 1..18: mol_type = other DNA
agagtttgatymtggctc

SEQ ID NO: 5 - DNA, 20 bp, synthetic construct
  misc_feature 1..20: note = Primer
  source 1..20: mol_type = other DNA
cggttaccttgttacgactt

SEQ ID NO: 6 - DNA, 19 bp, synthetic construct
  misc_feature 1..19: note = Primer
  source 1..19: mol_type = other DNA
gtgccagcmgccgcggtaa